European Patent Specification EP 3 578 655 B1, published April 10, 2024. Title: Nucleic acids for simultaneous inhibition of mTOR gene and STAT3 gene. Applicant: Curigene Co., Ltd. The sequence listing filed with the application follows.

SEQUENCE LISTING (25 sequences)

SEQ ID NO: 1 - RNA, 21 nt, Artificial Sequence
  antisense_mTOR of set 1
gactgtggcatccacctgcat

SEQ ID NO: 2 - RNA, 21 nt, Artificial Sequence
  antisense_STAT3 of set 1
atgcaggtaggcgcctcagtc

SEQ ID NO: 3 - RNA, 20 nt, Artificial Sequence
  antisense_mTOR of set 2
gactgtggcatccacctgca

SEQ ID NO: 4 - RNA, 20 nt, Artificial Sequence
  antisense_STAT3 of set 2
tgcaggtaggcgcctcagtc

SEQ ID NO: 5 - RNA, 19 nt, Artificial Sequence
  antisense_mTOR of set 3
gactgtggcatccacctgc

SEQ ID NO: 6 - RNA, 19 nt, Artificial Sequence
  antisense_STAT3 of set 3
gcaggtaggcgcctcagtc

SEQ ID NO: 7 - RNA, 18 nt, Artificial Sequence
  antisense_mTOR of set 4
gactgtggcatccacctg

SEQ ID NO: 8 - RNA, 18 nt, Artificial Sequence
  antisense_STAT3 of set 4
caggtaggcgcctcagtc

SEQ ID NO: 9 - RNA, 17 nt, Artificial Sequence
  antisense_mTOR of set 5
caagctgctgtggctga

SEQ ID NO: 10 - RNA, 17 nt, Artificial Sequence
  antisense_STAT3 of set 5
tcagctacagcagcttg

SEQ ID NO: 11 - RNA, 20 nt, Artificial Sequence
  antisense_mTOR of set 6
tgctgggccgcatgcgctgc

SEQ ID NO: 12 - RNA, 20 nt, Artificial Sequence
  antisense_STAT3 of set 6
gcagccactgcggcccagca

SEQ ID NO: 13 - RNA, 19 nt, Artificial Sequence
  antisense_mTOR of set 7
gctgggccgcatgcgctgc

SEQ ID NO: 14 - RNA, 19 nt, Artificial Sequence
  antisense_STAT3 of set 7
gcagccactgcggcccagc

SEQ ID NO: 15 - RNA, 18 nt, Artificial Sequence
  antisense_mTOR of set 8
ctgggccgcatgcgctgc

SEQ ID NO: 16 - RNA, 18 nt, Artificial Sequence
  antisense_STAT3 of set 8
gcagccactgcggcccag

SEQ ID NO: 17 - RNA, 17 nt, Artificial Sequence
  antisense_mTOR of set 9
tgggccgcatgcgctgc

SEQ ID NO: 18 - RNA, 17 nt, Artificial Sequence
  antisense_STAT3 of set 9
gcagccactgcggccca

SEQ ID NO: 19 - DNA, 276 bp, Artificial Sequence
  U7 promotor
cctagagtcgacactagataacaacataggagctgtgattggctgttttcagccaatcagcactgactcatttgcatagcctttacaagcggtcacaaactcaagaaacgagcggttttaatagtcttttagaatattgtttatcgaaccgaataaggaactgtgctttgtgattcacatatcagtggaggggtgtggaaatggcaccttgatctcaccctcatcgaaagtggagttgatgtccttccctggctcgctacagacgcacttccgcaa

SEQ ID NO: 20 - RNA, 54 nt, Artificial Sequence
  TTGGATCCAA loop shRNA
gactgtggcatccacctgcatttggatccaaatgcaggtaggcgcctcagtctt

SEQ ID NO: 21 - RNA, 54 nt, Artificial Sequence
  TTCAAGAGAG loop shRNA
gactgtggcatccacctgcatttcaagagagatgcaggtaggcgcctcagtctt

SEQ ID NO: 22 - RNA, 21 nt, Artificial Sequence
  antisense_mTOR
gactgtggcatccacctgcat

SEQ ID NO: 23 - RNA, 21 nt, Artificial Sequence
  antisense_STAT3
atgcaggtaggcgcctcagtc

SEQ ID NO: 24 - RNA, 23 nt, Artificial Sequence
  mTOR siRNA_sense strand
guggaaacaggacccaugadtdt

SEQ ID NO: 25 - RNA, 23 nt, Artificial Sequence
  STAT3 siRNA_sense strand
ucauggguccuguuuccacdtdt